European Patent Specification EP 3 690 055 B1, published December 11, 2024. Title: Labeling and treatment method of  tumorigenesis-causing cells in stem cells. Applicant: Kagoshima University. The sequence listing filed with the application follows.

SEQUENCE LISTING (18 sequences)

SEQ ID NO: 1 - DNA, 28 bp, Artificial Sequence
  primer
accggtcaccatggtgagggagctgatt

SEQ ID NO: 2 - DNA, 28 bp, Artificial Sequence
  primer
agatcttctgtgccccagtttgctaggg

SEQ ID NO: 3 - DNA, 30 bp, Artificial Sequence
  primer
accggtcaccatggtgagcaagggcgagga

SEQ ID NO: 4 - DNA, 30 bp, Artificial Sequence
  primer
ggatcccttgtacagctcgtccatgccgag

SEQ ID NO: 5 - DNA, 30 bp, Artificial Sequence
  primer
ggatccatggcttcgtaccccggccatcaa

SEQ ID NO: 6 - DNA, 30 bp, Artificial Sequence
  primer
gtttaaactcagttagcctcccccatctcc

SEQ ID NO: 7 - DNA, 30 bp, Artificial Sequence
  primer
ggatccatggcggcccggcgcggggctctc

SEQ ID NO: 8 - DNA, 29 bp, Artificial Sequence
  primer
cccgggtacctcacttccatagctccccc

SEQ ID NO: 9 - DNA, 35 bp, Artificial Sequence
  primer
ttctacgcgtaccggtgccatgctcgagggagtgc

SEQ ID NO: 10 - DNA, 22 bp, Artificial Sequence
  primer
gggcccgggattttcctccacg

SEQ ID NO: 11 - DNA, 35 bp, Artificial Sequence
  primer
gaaaatcccgggcccatggtgagcaagggcgagga

SEQ ID NO: 12 - DNA, 35 bp, Artificial Sequence
  primer
tggtcttaaaggtaccttacttgtacagctcgtcc

SEQ ID NO: 13 - DNA, 36 bp, Artificial Sequence
  primer
gaaaatcccgggcccatggtgagcgagctgattaag

SEQ ID NO: 14 - DNA, 36 bp, Artificial Sequence
  primer
tggtcttaaaggtacctcatctgtgccccagtttgc

SEQ ID NO: 15 - DNA, 26 bp, Artificial Sequence
  primer
cacctaaagtgaaatgaggtaaagcc

SEQ ID NO: 16 - DNA, 22 bp, Artificial Sequence
  primer
ggaaagatcatagaaagaagag

SEQ ID NO: 17 - DNA, 25 bp, Artificial Sequence
  primer
caccgaattctaccgggtaggggag

SEQ ID NO: 18 - DNA, 20 bp, Artificial Sequence
  primer
ctgcaggtcgaaaggcccgg